European Patent Application EP 4 296 360 A1, published December 27, 2023. Title: Protein having modified alpha-1,2-fucosyltransferase activity and method for producing fucose-containing saccharides. Applicant: KYOWA HAKKO BIO CO., LTD. The sequence listing filed with the application follows.

SEQUENCE LISTING (54 sequences)

SEQ ID NO: 1 - DNA, 861 bp, Helicobacter mustelae
atggattttaagattgtgcaagtgcatggaggacttggaaatcagatgtttcaatacgcttttgccaagagtttgcaaacacatctcaatatacccgtgctacttgataccacctggtttgattatggcaatcgggaattgggattgcatctttttcccatcgatttgcaatgtgctagtgcacagcaaattgctgctgcccatatgcaaaacctgccaaggctagtgagaggtgcgctcagacgtatgggtctaggcagagtcagcaaggaaatcgtgtttgaatacatgccagagctgtttgagccaagtcgcattgcttattttcatggctatttccaagatccaagatattttgaagacatctctcccctgattaagcaaacattcaccctgcctcaccccacagagcatgcagagcaatatagccgcaaactctctcagattttggcggcaaaaaatagcgtatttgtgcatataaggcgaggggattatatgagacttggctggcaacttgatatcagctaccaactacgcgccattgcatatatggccaagcgcgtgcaaaatttggagctatttttattttgcgaggatttggaatttgtgcagaatcttgatcttggctatccctttgtggatatgaccacaagggatggggcggcgcattgggatatgatgctgatgcaatcttgcaagcatggcattatcacaaatagtacctatagttggtgggcggcatatttgataaaaaatccagaaaaaatcattattggaccaagccactggatctatggcaatgaaaatatcctttgcaaggattgggtgaagatagaatcccaatttgagacaaaatcttga

SEQ ID NO: 2 - protein, 286 aa, Helicobacter mustelae
MDFKIVQVHGGLGNQMFQYAFAKSLQTHLNIPVLLDTTWFDYGNRELGLHLFPIDLQCASAQQIAAAHMQNLPRLVRGALRRMGLGRVSKEIVFEYMPELFEPSRIAYFHGYFQDPRYFEDISPLIKQTFTLPHPTEHAEQYSRKLSQILAAKNSVFVHIRRGDYMRLGWQLDISYQLRAIAYMAKRVQNLELFLFCEDLEFVQNLDLGYPFVDMTTRDGAAHWDMMLMQSCKHGIITNSTYSWWAAYLIKNPEKIIIGPSHWIYGNENILCKDWVKIESQFETKS

SEQ ID NO: 3 - DNA, 897 bp, Helicobacter pylori
atggcttttaaggtggtgcaaatttgcggggggcttgggaatcaaatgttccaatacgctttcgctaaaagtttgcaaaaacaccttaatacgcccgtgctattggatatcacttcttttgattggagtaataggaaaatgcaattagaacttttccctattgatttgccctatgcgagcgcgaaagaaatcgctatagctaaaatgcaacacctccccaagctagtaagagatacgctcaaatgcatggggtttgatagggtgagtcaagaaatcgtttttgaatacgagcctggattgttaaagccaagccgcttgacttatttttatggctattttcaagatccacgatattttgatgctatatcccctttaatcaagcaaaccttcaccctacccccccccgaaaatggaaataataaaaaaaaagaggaagaataccaccgcaagcttgctttgattttagccgctaaaaacagcgtgtttgtgcatgtaagaagaggggattatgtggggattggctgtcagcttggtattgattatcaaaaaaaggcgcttgagtatatagcaaagcgcgtgccaaacatggagctttttgtgttttgcgaagacttaaaattcacgcaaaatcttgatcttggctacccttttatggacatgaccactagggataaagaagaagaggcgtattgggacatgctgctcatgcaatcttgcaagcatggcattatcgctaacagcacttatagctggtgggcggcctatttgataaacaatccagaaaaaatcattattggccccaaacactggctttttgggcatgagaatatcctttgtaaggaatgggtgaaaatagaatcccattttgaggtaaaatcaaaaaaatataatgcttaa

SEQ ID NO: 4 - protein, 296 aa, Helicobacter pylori
MAFKVVQICGGLGNQMFQYAFAKSLQKHLNTPVLLDTTSFDWSNRKMQLELFPIDLPYASEKEIAIAKMQHLPKLVREALKCMGFDRVSKEIVFEYEPKLLKPSRLTYFYGYFQDPRYFDAISPLIKQTFTLPPPENNKKKEEEYHRKLSLILAAKNSVFVHIRRGDYVGIGCQLGIDYQKKAVGYMAKRVPNMELFVFCEDLEFTQNLDLGYPFMDMTTRDKEEEGYWDMLLMQSCKHGIIANSTYSWWAAYLINNPEKIIIGPKHWLFGHENILCKEWVKIESHFEVKSQKYNA

SEQ ID NO: 5 - DNA, 894 bp, Escherichia coli
atgtctattataagattacaaggcggacttggaaatcaactttttcagttctcatttgggtatgcgctttccaaaattaatgggacaccattatattttgatataagtcattatgctgaaaatgatgatcatggtggttacaggctaaacaatctacaaattccagaggaatatttacagtattacacaccaaaaattaataatatttataaatttttggttcgtgggtcaagattatatcctgaaatctttctttttttaggtttttgcaatgaatttcatgcctatggttatgattttgaatatatagcgcaaaaatggaaatccaaaaaatatatagggtattggcaatctgagcactttttccataaacatatattagatctaaaagaattttttattccaaagaatgtgtctgaacaagcaaatttacttgcagcaaaaattcttgaatctcaatcatcactttctattcatataagaagaggagattatataaaaaacaaaacagctactttaactcatggcgtttgttcgttagagtattacaaaaaagctttaaataaaatacgcgatttggcaatgatacgtgacgtgtttattttcagtgatgatattttttggtgtaaagaaaatatcgaaacattactcagtaaaaaatataatatatattattcagaagatttatcacaagaagaagatttatggttaatgagcttagctaaccatcatattatagcgaatagtagttttagttggtggggggcttatttaggtacatcagcgtcacagattgttatttatcctactccttggtacgatataactccaaaaaatacttatatccccatagtcaatcactggataaacgtggataaacatagctcgtgttag

SEQ ID NO: 6 - protein, 297 aa, Escherichia coli
MSIIRLQGGLGNQLFQFSFGYALSKINGTPLYFDISHYAENDDHGGYRLNNLQIPEEYLQYYTPKINNIYKFLVRGSRLYPEIFLFLGFCNEFHAYGYDFEYIAQKWKSKKYIGYWQSEHFFHKHILDLKEFFIPKNVSEQANLLAAKILESQSSLSIHIRRGDYIKNKTATLTHGVCSLEYYKKALNKIRDLAMIRDVFIFSDDIFWCKENIETLLSKKYNIYYSEDLSQEEDLWLMSLANHHIIANSSFSWWGAYLGTSASQIVIYPTPWYDITPKNTYIPIVNHWINVDKHSSC

SEQ ID NO: 7 - DNA, 864 bp, Bacteroides fragilis
atgttatatgtaattttacgtggacgattaggtaataatctttttcagatagcaactgccgcttcgttgactcagaattttatattttgtacagtaaataaggaccaagagagacaggtccttttgtataaggattctttttttaaaaatataaaagttatgaagggggttcctgatggcataccatattacaaagaaccattccatgaatttagcagaattccttatgaagaaggaaaggatctcattattgatggatatttccaatcagaaaagtactttaaaagaagtgtcgtattagatctttatagaataactgatgagctaaggaagaaaatatggaatatttgtggaaatattttagaaaagggagaaactgtgagtattcatgttagaagaggtgattacttgaagctgccacatgcattaccattttgtggaaagtcatactataagaatgctattcaatatattggtgaggataaaatattcattatttgtagtgatgatatcgattggtgtaaaaaaaactttataggaaaaagatattacttcatagagaacactactcctttactagatttatatatccaatccttgtgcactcacaatattataagtaatagctcttttagttggtggggagcatggcttaatgaaaatagtaataaaattgttattgcacctcaaatgtggtttggcatttctgtgaagttgggtgttagtgatttattgcctgtcagttgggttcgacttcctaataattatactttaggaagatattgttttgctctatataaagtagttgaggactatttattaaatattctgcgattaatatggaaaagaaagaagaatatgtga

SEQ ID NO: 8 - protein, 288 aa, Bacteroides fragilis
MLYVILRGRLGNNLFQIATAASLTQNFIFCTVNKDQERQVLLYKDSFFKNIKVMKGVPDGIPYYKEPFHEFSRIPYEEGKDLIIDGYFQSEKYFKRSVVLDLYRITDELRKKIWNICGNILEKGETVSIHVRRGDYLKLPHALPFCGKSYYKNAIQYIGEDKIFIICSDDIDWCKKNFIGKRYYFIENTTPLLDLYIQSLCTHNIISNSSFSWWGAWLNENSNKIVIAPQMWFGISVKLGVSDLLPVSWVRLPNNYTLGRYCFALYKVVEDYLLNILRLIWKRKKNMG

SEQ ID NO: 9 - DNA, 846 bp, Vibrio cholerae
atgatcgttatgaaaatatcgggtggcttaggcaatcaattgtttcagtacgctgtgggtagggcaatagccattcaatatggtgttccattaaaattggatgttagtgcttataaaaattataagctccataatggctaccgattagatcagtttaatattaatgccgatatagcgaatgaggatgaaatttttcatttgaaaggttccagtaatcgtttgtctagaattttaagacgattaggttggttgaagaaaaacacgtattacgctgaaaaacaaagaacgatttatgatgttagtgttttcatgcaagcaccacgctatttagatggttattggcaaaatgagcaatatttttcacagataagagcggtattactgcaagaactctggccaaatcaacctttaagcattaacgcgcaagctcatcagataaaaattcagcagactcatgctgtcagtattcatgttagaagaggggattatttgaatcaccctgaaattggagttcttgatatagactactataaacgtgctgttgactatataaaggaaaaaattgaagcgccagtattttttgtgttttctaatgatgtagcatggtgcaaagataatttcaattttattgatagcccagtctttattgaagacacacaaacagaaattgacgatctaatgctgatgtgccagtgtcaacataatattgttgcaaacagttcttttagttggtgggctgcttggttaaatagtaatgttgataagattgttattgcccctaaaacgtggatggctgaaaatccaaaaggctataaatgggtacctgattcatggcgtgaaatatga

SEQ ID NO: 10 - protein, 280 aa, Vibrio cholerae
MIVMKISGGLGNQLFQYAVGRAIAIQYGVPLKLDVSAYKNYKLHNGYRLDQFNINADIANEDEIFHLKGSSNRLSRILRRLGWLKKNTYYAEKQRTIYDVSVFMQAPRYLDGYWQNEQYFSQIRAVLLQELWPNQPLSINAQAHQIKIQQTHAVSIHVRRGDYLNHPEIGVLDIDYYKRAVDYIKEKIEAPVFFVFSNDVAWCKDNFNFIDSPVFIEDTQTEIDDLMLMCQCQHNIVANSSFSWWAAWLNSNVDKIVIAPKTWMAENPKGYKWVPDSWRE

SEQ ID NO: 11 - DNA, 861 bp, Artificial Sequence
  Synthetic DNA
atggattttaagattgtgcaagtgcgcggaggacttggaaatcagatgtttcaatacgcttttgccaagagtttgcaaacacatctcaatatacccgtgctacttgataccacctggtttgattatggcaatcgggaattgggattgcatctttttcccatcgatttgcaatgtgctagtgcacagcaaattgctgctgcccgcatgcaaaacctgccaaggcccgtgagaggtgcgctcagacgtatgggtctaagtagagtcagcaaggaaatcgtgtttgaatacatgccagagctgtttgagccaagtcgcattgcttattttcatggctatttccaagatccaagatattttgaagacatctctcccctgattaagcaaacattcaccctgcctcaccccacagagcatgcagagcaatatagccgcaaactctctcagattttggcggcaaaaaatagcgtatttgtgcatataaggcgaggggattatatgagacttggctggcaacttgatatcagctaccaactacgcgccattgcatatatggccaagcgcgtgcaaaatttggagctatttttattttgcgaggatttggaatttgtgcagaatcttgatcttggctatccctttgtggatatgaccacaagggatggggcggcgcattgggatatgatgctgatgcaatcttgcaagcatggcattatcgctaatagtacctatagttggtgggcggcatatttgataaaaaatccagaaaaaatcattattggaccaagccactggatctatggcaatgaaaatatcctttgcaaggattgggtgaagatagaatcccaatttgagacaaaatcttga

SEQ ID NO: 12 - DNA, 861 bp, Artificial Sequence
  Synthetic DNA
atggattttaagattgtgcaagtgcgcggaggacttggaaatcagatgtttcaatacgcttttgccaagagtttgcaaacacatctcaatatacccgtgctacttgataccacctggtttgattatggcaatcgggaattgggattgcatctttttcccatcgatttgcaatgtgctagtgcacagcaaattgctgctgcccatatgcaaaacctgccaaggctagtgagaggtgcgctcagacgtatgggtctaggcagagtcagcaaggaaatcgtgtttgaatacatgccagagctgtttgagccaagtcgcattgcttattttcatggctatttccaagatccaagatattttgaagacatctctcccctgattaagcaaacattcaccctgcctcaccccacagagcatgcagagcaatatagccgcaaactctctcagattttggcggcaaaaaatagcgtatttgtgcatataaggcgaggggattatatgagacttggctggcaacttgatatcagctaccaactacgcgccattgcatatatggccaagcgcgtgcaaaatttggagctatttttattttgcgaggatttggaatttgtgcagaatcttgatcttggctatccctttgtggatatgaccacaagggatggggcggcgcattgggatatgatgctgatgcaatcttgcaagcatggcattatcacaaatagtacctatagttggtgggcggcatatttgataaaaaatccagaaaaaatcattattggaccaagccactggatctatggcaatgaaaatatcctttgcaaggattgggtgaagatagaatcccaatttgagacaaaatcttga

SEQ ID NO: 13 - DNA, 861 bp, Artificial Sequence
  Synthetic DNA
atggattttaagattgtgcaagtgcatggaggacttggaaatcagatgtttcaatacgcttttgccaagagtttgcaaacacatctcaatatacccgtgctacttgataccacctggtttgattatggcaatcgggaattgggattgcatctttttcccatcgatttgcaatgtgctagtgcacagcaaattgctgctgcccatatgcaaaacctgccaaggctagtgagaggtgcgctcagacgtatgggtctaggcagagtcagcaaggaaatcgtgtttgaatacatgccagagctgtttgagccaagtcgcattgcttattttcatggctatttccaagatccaagatattttgaagacatctctcccctgattaagcaaacattcaccctgcctcaccccacagagcatgcagagcaatatagccgcaaactctctcagattttggcggcaaaaaatagcgtatttgtgcatataaggcgaggggattatatgagacttggctggcaacttgatatcagctaccaactacgcgccattgcatatatggccaagcgcgtgcaaaatttggagctatttttattttgcgaggatttggaatttgtgcagaatcttgatcttggctatccctttgtggatatgaccacaagggatggggcggcgcattgggatatgatgctgatgcaatcttgcaagcatggcattatcgctaatagtacctatagttggtgggcggcatatttgataaaaaatccagaaaaaatcattattggaccaagccactggatctatggcaatgaaaatatcctttgcaaggattgggtgaagatagaatcccaatttgagacaaaatcttga

SEQ ID NO: 14 - DNA, 861 bp, Artificial Sequence
  Synthetic DNA
atggattttaagattgtgcaagtgcgcggaggacttggaaatcagatgtttcaatacgcttttgccaagagtttgcaaacacatctcaatatacccgtgctacttgataccacctggtttgattatggcaatcgggaattgggattgcatctttttcccatcgatttgcaatgtgctagtgcacagcaaattgctgctgcccatatgcaaaacctgccaaggctagtgagaggtgcgctcagacgtatgggtctaggcagagtcagcaaggaaatcgtgtttgaatacatgccagagctgtttgagccaagtcgcattgcttattttcatggctatttccaagatccaagatattttgaagacatctctcccctgattaagcaaacattcaccctgcctcaccccacagagcatgcagagcaatatagccgcaaactctctcagattttggcggcaaaaaatagcgtatttgtgcatataaggcgaggggattatatgagacttggctggcaacttgatatcagctaccaactacgcgccattgcatatatggccaagcgcgtgcaaaatttggagctatttttattttgcgaggatttggaatttgtgcagaatcttgatcttggctatccctttgtggatatgaccacaagggatggggcggcgcattgggatatgatgctgatgcaatcttgcaagcatggcattatcgctaatagtacctatagttggtgggcggcatatttgataaaaaatccagaaaaaatcattattggaccaagccactggatctatggcaatgaaaatatcctttgcaaggattgggtgaagatagaatcccaatttgagacaaaatcttga

SEQ ID NO: 15 - DNA, 20 bp, Artificial Sequence
  Synthetic DNA
accaggcgtttaagggcacc

SEQ ID NO: 16 - DNA, 45 bp, Artificial Sequence
  Synthetic DNA
gactacgggcctaaagtcgacagaataaataaatcctggtgtccc

SEQ ID NO: 17 - DNA, 28 bp, Artificial Sequence
  Synthetic DNA
gtcgactttaggcccgtagtctgcaaat

SEQ ID NO: 18 - DNA, 21 bp, Artificial Sequence
  Synthetic DNA
tacggttagccatttgcctgc

SEQ ID NO: 19 - DNA, 44 bp, Artificial Sequence
  Synthetic DNA
ggtgcccttaaacgcctggtagctgtttcctgtgtgaaattgtt

SEQ ID NO: 20 - DNA, 19 bp, Artificial Sequence
  Synthetic DNA
tcgcgcaacgcgtcagtgg

SEQ ID NO: 21 - DNA, 44 bp, Artificial Sequence
  Synthetic DNA
gcaggcaaatggctaaccgtaatgaacatgtcgatgacagaaag

SEQ ID NO: 22 - DNA, 20 bp, Artificial Sequence
  Synthetic DNA
tgcgctgtgtgtcgttgggc

SEQ ID NO: 23 - DNA, 45 bp, Artificial Sequence
  Synthetic DNA
ttctgtcatcgacatgttcatagctgtttcctgtgtgaaattgtt

SEQ ID NO: 24 - DNA, 23 bp, Artificial Sequence
  Synthetic DNA
atgaacatgtcgatgacagaaag

SEQ ID NO: 25 - DNA, 42 bp, Artificial Sequence
  Synthetic DNA
ggtgcccttaaacgcctggtcgttgttcctgttatttgcccc

SEQ ID NO: 26 - DNA, 21 bp, Artificial Sequence
  Synthetic DNA
aagctggtgattaactccggg

SEQ ID NO: 27 - DNA, 44 bp, Artificial Sequence
  Synthetic DNA
gcaggcaaatggctaaccgtaatttgcgaccattcctggaaaaa

SEQ ID NO: 28 - DNA, 20 bp, Artificial Sequence
  Synthetic DNA
gcacatagcgaccaacggcc

SEQ ID NO: 29 - DNA, 45 bp, Artificial Sequence
  Synthetic DNA
tttttccaggaatggtcgcaaatcgttgttcctgttatttgcccc

SEQ ID NO: 30 - DNA, 23 bp, Artificial Sequence
  Synthetic DNA
atttgcgaccattcctggaaaaa

SEQ ID NO: 31 - DNA, 26 bp, Artificial Sequence
  Synthetic DNA
atgtcaacgattattatggatttatg

SEQ ID NO: 32 - DNA, 45 bp, Artificial Sequence
  Synthetic DNA
atccattctagacctccttaattagcgcatgttgacaaaaatacc

SEQ ID NO: 33 - DNA, 39 bp, Artificial Sequence
  Synthetic DNA
ttaaggaggtctagaatggattttaagattgtgcaagtg

SEQ ID NO: 34 - DNA, 45 bp, Artificial Sequence
  Synthetic DNA
cataatggatttcctctcgagtcaagattttgtctcaaattggga

SEQ ID NO: 35 - DNA, 45 bp, Artificial Sequence
  Synthetic DNA
ctcgagaggaaatccattatgtactatttaaaaaacacaaacttt

SEQ ID NO: 36 - DNA, 23 bp, Artificial Sequence
  Synthetic DNA
ttaagcgacttcattcacctgac

SEQ ID NO: 37 - DNA, 41 bp, Artificial Sequence
  Synthetic DNA
gaggagaaattaaccatgtcaacgattattatggatttatg

SEQ ID NO: 38 - DNA, 38 bp, Artificial Sequence
  Synthetic DNA
agggcatcggtcgacttaagcgacttcattcacctgac

SEQ ID NO: 39 - DNA, 21 bp, Artificial Sequence
  Synthetic DNA
gtcgaccgatgcccttgagag

SEQ ID NO: 40 - DNA, 25 bp, Artificial Sequence
  Synthetic DNA
ggttaatttctcctctttaatatcg

SEQ ID NO: 41 - DNA, 27 bp, Artificial Sequence
  Synthetic DNA
caagtgcgcggaggacttggaaatcag

SEQ ID NO: 42 - DNA, 27 bp, Artificial Sequence
  Synthetic DNA
tcctccgcgcacttgcacaatcttaaa

SEQ ID NO: 43 - DNA, 27 bp, Artificial Sequence
  Synthetic DNA
gctgcccgcatgcaaaacctgccaagg

SEQ ID NO: 44 - DNA, 27 bp, Artificial Sequence
  Synthetic DNA
ttgcatgcgggcagcagcaatttgctg

SEQ ID NO: 45 - DNA, 27 bp, Artificial Sequence
  Synthetic DNA
ccaaggcccgtgagaggtgcgctcaga

SEQ ID NO: 46 - DNA, 27 bp, Artificial Sequence
  Synthetic DNA
tctcacgggccttggcaggttttgcat

SEQ ID NO: 47 - DNA, 27 bp, Artificial Sequence
  Synthetic DNA
ggtctaagtagagtcagcaaggaaatc

SEQ ID NO: 48 - DNA, 27 bp, Artificial Sequence
  Synthetic DNA
gactctacttagacccatacgtctgag

SEQ ID NO: 49 - DNA, 27 bp, Artificial Sequence
  Synthetic DNA
attatcgctaatagtacctatagttgg

SEQ ID NO: 50 - DNA, 27 bp, Artificial Sequence
  Synthetic DNA
actattagcgataatgccatgcttgca

SEQ ID NO: 51 - protein, 286 aa, Artificial Sequence
  Synthetic Protein
MDFKIVQVRGGLGNQMFQYAFAKSLQTHLNIPVLLDTTWFDYGNRELGLHLFPIDLQCASAQQIAAARMQNLPRPVRGALRRMGLSRVSKEIVFEYMPELFEPSRIAYFHGYFQDPRYFEDISPLIKQTFTLPHPTEHAEQYSRKLSQILAAKNSVFVHIRRGDYMRLGWQLDISYQLRAIAYMAKRVQNLELFLFCEDLEFVQNLDLGYPFVDMTTRDGAAHWDMMLMQSCKHGIIANSTYSWWAAYLIKNPEKIIIGPSHWIYGNENILCKDWVKIESQFETKS

SEQ ID NO: 52 - protein, 286 aa, Artificial Sequence
  Synthetic Protein
MDFKIVQVRGGLGNQMFQYAFAKSLQTHLNIPVLLDTTWFDYGNRELGLHLFPIDLQCASAQQIAAAHMQNLPRLVRGALRRMGLGRVSKEIVFEYMPELFEPSRIAYFHGYFQDPRYFEDISPLIKQTFTLPHPTEHAEQYSRKLSQILAAKNSVFVHIRRGDYMRLGWQLDISYQLRAIAYMAKRVQNLELFLFCEDLEFVQNLDLGYPFVDMTTRDGAAHWDMMLMQSCKHGIITNSTYSWWAAYLIKNPEKIIIGPSHWIYGNENILCKDWVKIESQFETKS

SEQ ID NO: 53 - protein, 286 aa, Artificial Sequence
  Synthetic Protein
MDFKIVQVHGGLGNQMFQYAFAKSLQTHLNIPVLLDTTWFDYGNRELGLHLFPIDLQCASAQQIAAAHMQNLPRLVRGALRRMGLGRVSKEIVFEYMPELFEPSRIAYFHGYFQDPRYFEDISPLIKQTFTLPHPTEHAEQYSRKLSQILAAKNSVFVHIRRGDYMRLGWQLDISYQLRAIAYMAKRVQNLELFLFCEDLEFVQNLDLGYPFVDMTTRDGAAHWDMMLMQSCKHGIIANSTYSWWAAYLIKNPEKIIIGPSHWIYGNENILCKDWVKIESQFETKS

SEQ ID NO: 54 - protein, 286 aa, Artificial Sequence
  Synthetic Protein
MDFKIVQVRGGLGNQMFQYAFAKSLQTHLNIPVLLDTTWFDYGNRELGLHLFPIDLQCASAQQIAAAHMQNLPRLVRGALRRMGLGRVSKEIVFEYMPELFEPSRIAYFHGYFQDPRYFEDISPLIKQTFTLPHPTEHAEQYSRKLSQILAAKNSVFVHIRRGDYMRLGWQLDISYQLRAIAYMAKRVQNLELFLFCEDLEFVQNLDLGYPFVDMTTRDGAAHWDMMLMQSCKHGIIANSTYSWWAAYLIKNPEKIIIGPSHWIYGNENILCKDWVKIESQFETKS